European Patent Application EP 4 273 549 A1, published November 8, 2023. Title: PROTEIN BINDING DOMAINS STABILIZING FUNCTIONAL CONFORMATIONAL STATES OF GPCRS. Applicant: VIB VZW. The sequence listing filed with the application follows.

SEQUENCE LISTING (73 sequences)

SEQ ID NO: 1 - protein, 120 aa, Lama glama
QVQLQESGGGLVQAGGSLRLSCAASGSIFSINTMGWYRQAPGKQRELVAAIHSGGSTNYADSVKGRFTISRDNAKNTVYLQMNSLKPEDTAVYYCNVKDYGAVLYEYDYWGQGTQVTVSS

SEQ ID NO: 2 - protein, 120 aa, Lama glama
QVQLQESGGGLVQPGGSLRLSCAASGSIFSINTMGWYRQAPGKQRELVAAIHSGGSTNYANSVKGRFTISRDNAANTVYLQMNSLKPEDTAVYYCNVKDYGAVLYEYDYWGQGTQVTVSS

SEQ ID NO: 3 - protein, 120 aa, Lama glama
QVQLQESGGGLVQAGGSLRLSCAASGSIFSINTMGWYRQAPGKRRELVAAIHSGGSTNYANSVKGRFTISRDNAANTVYLQMNSLKPEDTAVYYCNVKDYGAVLYEYDYWGQGTQVTVSS

SEQ ID NO: 4 - protein, 120 aa, Lama glama
QVQLQESGGGLVQAGGSLRLSCAASGSIFSINTMGWYRQAPGKQRELVAAIHSGGSTNYANSVKGRFTISRDNAANTVYLQMNSLKPEDTAVYYCNVKDYGAVLYEYDYWGQGTQVTVSS

SEQ ID NO: 5 - protein, 120 aa, Lama glama
QVQLQESGGGLVQAGGSLRLSCAASGSIFSINTMGWYRQAPGKQRELVAAIHSGGSTNYADSVRGRFTISRDNAKNTVYLQMNSLKPEDTAVYYCNVKDYGAVLYEYDYWGQGTQVTVSS

SEQ ID NO: 6 - protein, 119 aa, Lama glama
QVQLQESGGGLVQAGGSLRLSCAASGSIFSLNDMGWYRQAPGKQRELVAAITSGGSTNYADSVKGRFTISRDNAKNTVYLQMNSLKPEDTAVYYCNAVVAGTFSTYDYWGQGTQVTVSS

SEQ ID NO: 7 - protein, 119 aa, Lama glama
QVQLQESGGGLVQAGGPLRLSCAASGSIFSLNDMGWYRQAPGKQRELVAAITSGGSTNYADSVKGRFTISRDNAKNTVYLQMNSLKPEDTAVYYCNAVVAGTFSTYDYWGQGTQVTVSS

SEQ ID NO: 8 - protein, 119 aa, Lama glama
QVQLQESGGGLVQAGGSLRLSCAASGSIFSLNDMGWYRQAPGKQRELVAAISSGGRLNYADSVKGRFTISRDNAKNTVYLQMNSLKPEDTAVYYCNAVVAGTFSTYDYWGQGTQVTVSS

SEQ ID NO: 9 - protein, 119 aa, Lama glama
QVQLQESGGGLVQPGGSLRLSCAASGSIFSLNDMGWYRQAPGKQRELVAAISSGGRLNYADSVKGRFTISRDNAKNTVYLQMNSLKPEDTAVYYCNAVVAGTFSTYDYWGQGTQVTVSS

SEQ ID NO: 10 - protein, 119 aa, Lama glama
QVQLQESGGGLVQAGGSLRLSCAASGSIFSLNDMGWYRQAPGKQRDLVAAITSGGSTKYADSVKGRFTVSRDNAKNTVYLQMNSLKPEDTAVYYCNAKVAGTFSIYDYWGQGTQVTVSS

SEQ ID NO: 11 - protein, 119 aa, Lama glama
QVQLQESGGGLVQAGGSLRLSCAASGSIFSLNDMGWYRQAPGKLRELVAAVTSGGSTNYADSVKGRFTISRDNAKNTVYLQMNSLKPEDTAVYYCNAKVAGTFSIYDYWGQGTQVTVSS

SEQ ID NO: 12 - protein, 119 aa, Lama glama
QVQLQESGGGLVQPGGSLRLSCAASGSIFSLNDMGWYRQAPGKLRELVAAITSGGSTKYADSVKGRFTISRDNAKNTVYLQMNSLKAEDTAVYYCNAKVAGTFSIYDYWGQGTQVTVSS

SEQ ID NO: 13 - protein, 119 aa, Lama glama
QVQLQESGGGLVQAGGSLRLSCAASGSIFSLNDMGWYRQAPGKLRELVAAITSGGSTKYADPVKGRFTISRDNAKNTVYLQMNSLKAEDTAVYYCNAKVAGTFSIYDYWGQGTQVTVSS

SEQ ID NO: 14 - protein, 119 aa, Lama glama
QVQLQESGGGLVQAGGSLRLSCAASGSIFSLNDMGWYRQAPGKLRELVAAITSGGSTKYADSVKGRFTISRDNAKNTVYLQMNSLKAEDTAVYYCNAKVAGTFSIYDYWGQGTQVTVSS

SEQ ID NO: 15 - protein, 119 aa, Lama glama
QVQLQESGGGLVQAGGSLRLSCAASGSIFSLNDMGWYRQAPGKQRELVAAITSGRSTNYADSVKGRFTISRDNAKNTVYLQMNSLKPEDTAVYYCNAKVAGTFSIYDYWGQGTQVTVSS

SEQ ID NO: 16 - protein, 119 aa, Lama glama
QVQLQESGGGLVQAGGSLRLSCAASGSIFSLNDMGWYRQAPGKQRELVAAITSGGSTNYADSVKGRFTISRDNAKNTVYLQMNSLKPEDTAVYYCNAKVAGTFSIYDYWGQGTQVTVSS

SEQ ID NO: 17 - protein, 119 aa, Lama glama
QVQLQESGGGLVQAGRSLRLSCAASGSIFSINDMGWFRQVPGKQRELVAAITSGGSVNYAEPVKGRFTISRDNGKNTVYLQMNSLKPEDTAVYYCNAKVAGTFSIYDYWGQGTQVTVSS

SEQ ID NO: 18 - protein, 119 aa, Lama glama
QVQLQESGGGLVQAGGSLRLSCAASGTIFSNNAMGWHRQAPGKQRELVAAITSGGSTNYADSVKGRFTISRDNAKNTVYLLMNSLKPEDTAVYYCNAKVPGTFSIYDYWGQGTQVTVSS

SEQ ID NO: 19 - protein, 115 aa, Lama glama
QVQLQESGGGLVQAGGSLRLSCAASGSVFSLPTAGWYRQAPGKQRELVALITGSGSTHYADSVKGRFAISREYSKKTMDLQMNSLHREDTAVYFCYYRSTFTEYWGQGTQVTVSS

SEQ ID NO: 20 - protein, 120 aa, Lama glama
QVQLQESGGGLVQAGGSLRLSCAASGTISSFIAMGWYRQSPGKQRELVAGITSGGETNYEDSVKGRFTISRDNAKNTLYLQMNTLKPEDTAVYYCNAQVFADIFNLINYWGQGTQVTVSS

SEQ ID NO: 21 - protein, 118 aa, Lama glama
QVQLQESGGGLVQAGGSLRLSCAASGTIFSPNTMAWYRQAPGKQRELVALITSGGSRNYADYVKGRFTISRDNAKNTLYLQMNNLKPEDTAVYYCNYQTVFFGNAEAWGQGTQVTVSS

SEQ ID NO: 22 - protein, 122 aa, Lama glama
QVQLQESGGGLVQAGGSLRLSCAASGSIFSINAMGWYRQAPGKQRELVAASTSGDITNYADSVKGRFTISRDNAKNTVYLQMNSLEPEDTGVYYCNARGIYSDYAFADFNSWGQGTQVTVSS

SEQ ID NO: 23 - protein, 114 aa, Lama glama
QVQLQESGGGLVQAGGSLRLSCASSGSRFSFITMGWLRQAPGKQRELVATLSGDNTNYSDAVKGRFTISRDNARNTVYLQMNGLKPEDTGTYYCRGTSVLYDVWGQGTQVTVSS

SEQ ID NO: 24 - protein, 124 aa, Lama glama
QVQLQESGGGLVQPGGSLRLSCAASGFTFSGYAMNWVRQAPGKGPEWVSAINSGGGSTSYADSVKGRFTISRDNAKNTVYLQMNSLKPEDTAVYYCHARDIYSDFLGQYEYDYWGQGTQVTVSS

SEQ ID NO: 25 - protein, 116 aa, Lama glama
QVQLQESGGGLVQPGGSLRLSCAASGFAFSSYELRWYRQAPGKQHELVAGITTGGNTYYADSVKGRFTISRDNAKNTVYLQMSNLRPEDTAVYACNANWDLLSDYWGQGTQVTVSS

SEQ ID NO: 26 - protein, 123 aa, Lama glama
QVQLQESGGGLVQPGGSLRLSCAASGSIFSINAMGWYRQAPGKQRDLVASITSGGSTNYADSVKGRFTISRDNAKNTVYLQMNSLKPEDTAVYYCNVQGTGPSSWLFNEYDYWGQGTQVTVSS

SEQ ID NO: 27 - protein, 123 aa, Lama glama
QVQLQESGGGLVQPGGSLGLSCAASGSIFSINSMGWYRQAPGKQRELVAAITSDGSTNYADSVKGRFTISRDNAKNTVYLQMNSLKPEDTAVYVCNADSVYSDFLGKYEYDYWGQGTQVTVSS

SEQ ID NO: 28 - protein, 123 aa, Lama glama
QVQLQESGGGLVQPGGSLRLSCAASGSIFSLNAMRWYRQAPGKQRELVAAITSDGSTNYADSVKGRFTISRDNAKNTVYLQMNSLKPEDTAVYYCNADSVYSDFLGKYEYDYWGQGTQVTVSS

SEQ ID NO: 29 - protein, 123 aa, Lama glama
QVQLQESGGGLVQAGGSLRLSCAASGSIFSINAMGWYRQAPGKQRELVAAITSGGSTTYADSVKGRFTVSRDNAKNTVYLQMIRLKPEDTAVYYCHVRDIYSDFLGQYEYDYWGQGTQVTVSS

SEQ ID NO: 30 - protein, 8 aa, Lama glama
GSIFSINT

SEQ ID NO: 31 - protein, 8 aa, Lama glama
GSIFSLND

SEQ ID NO: 32 - protein, 8 aa, Lama glama
GSIFSIND

SEQ ID NO: 33 - protein, 8 aa, Lama glama
GTIFSNNA

SEQ ID NO: 34 - protein, 8 aa, Lama glama
GSVFSLPT

SEQ ID NO: 35 - protein, 8 aa, Lama glama
GTISSFIA

SEQ ID NO: 36 - protein, 8 aa, Lama glama
GTIFSPNT

SEQ ID NO: 37 - protein, 8 aa, Lama glama
GSIFSINA

SEQ ID NO: 38 - protein, 8 aa, Lama glama
GSRFSFIT

SEQ ID NO: 39 - protein, 8 aa, Lama glama
GFTFSGYA

SEQ ID NO: 40 - protein, 8 aa, Lama glama
GFAFSSYE

SEQ ID NO: 41 - protein, 8 aa, Lama glama
GSIFSINS

SEQ ID NO: 42 - protein, 8 aa, Lama glama
GSIFSLNA

SEQ ID NO: 43 - protein, 7 aa, Lama glama
IHSGGST

SEQ ID NO: 44 - protein, 7 aa, Lama glama
ITSGGST

SEQ ID NO: 45 - protein, 7 aa, Lama glama
ISSGGRL

SEQ ID NO: 46 - protein, 7 aa, Lama glama
VTSGGST

SEQ ID NO: 47 - protein, 7 aa, Lama glama
ITSGRST

SEQ ID NO: 48 - protein, 7 aa, Lama glama
ITSGGSV

SEQ ID NO: 49 - protein, 7 aa, Lama glama
ITGSGST

SEQ ID NO: 50 - protein, 7 aa, Lama glama
ITSGGET

SEQ ID NO: 51 - protein, 7 aa, Lama glama
ITSGGSR

SEQ ID NO: 52 - protein, 7 aa, Lama glama
STSGDIT

SEQ ID NO: 53 - protein, 6 aa, Lama glama
LSGDNT

SEQ ID NO: 54 - protein, 8 aa, Lama glama
INSGGGST

SEQ ID NO: 55 - protein, 7 aa, Lama glama
ITTGGNT

SEQ ID NO: 56 - protein, 7 aa, Lama glama
ITSDGST

SEQ ID NO: 57 - protein, 14 aa, Lama glama
NVKDYGAVLYEYDY

SEQ ID NO: 58 - protein, 13 aa, Lama glama
NAVVAGTFSTYDY

SEQ ID NO: 59 - protein, 13 aa, Lama glama
NAKVAGTFSIYDY

SEQ ID NO: 60 - protein, 13 aa, Lama glama
NAKVPGTFSIYDY

SEQ ID NO: 61 - protein, 9 aa, Lama glama
YYRSTFTEY

SEQ ID NO: 62 - protein, 14 aa, Lama glama
NAQVFADIFNLINY

SEQ ID NO: 63 - protein, 12 aa, Lama glama
NYQTVFFGNAEA

SEQ ID NO: 64 - protein, 16 aa, Lama glama
NARGIYSDYAFADFNS

SEQ ID NO: 65 - protein, 9 aa, Lama glama
RGTSVLYDV

SEQ ID NO: 66 - protein, 17 aa, Lama glama
HARDIYSDFLGQYEYDY

SEQ ID NO: 67 - protein, 10 aa, Lama glama
NANWDLLSDY

SEQ ID NO: 68 - protein, 17 aa, Lama glama
NVQGTGPSSWLFNEYDY

SEQ ID NO: 69 - protein, 17 aa, Lama glama
NADSVYSDFLGKYEYDY

SEQ ID NO: 70 - protein, 17 aa, Lama glama
HVRDIYSDFLGQYEYDY

SEQ ID NO: 71 - protein, 11 aa, synthetic construct
  REGION 1..11: note = HIV-derived TAT peptide
YGRKKRRQRRR

SEQ ID NO: 72 - protein, 477 aa, Homo sapiens
MGAGVLVLGASEPGNLSSAAPLPDGAATAARLLVPASPPASLLPPASESPEPLSQQWTAGMGLLMALIVLLIVAGNVLVIVAIAKTPRLQTLTNLFIMSLASADLVMGLLVVPFGATIVVWGRWEYGSFFCELWTSVDVLCVTASIETLCVIALDRYLAITSPFRYQSLLTRARARGLVCTVWAISALVSFLPILMHWWRAESDEARRCYNDPKCCDFVTNRAYAIASSVVSFYVPLCIMAFVYLRVFREAQKQVKKIDSCERRFLGGPARPPSPSPSPVPAPAPPPGPPRPAAAAATAPLANGRAGKRRPSRLVALREQKALKTLGIIMGVFTLCWLPFFLANVVKAFHRELVPDRLFVFFNWLGYANSAFNPIIYCRSPDFRKAFQRLLCCARRAARRRHATHGDRPRASGCLARPGPPPSPGAASDDDDDDVVGATPPARLLEPWAGCNGGAAADSDSSLDEPCRPGFASESKV

SEQ ID NO: 73 - protein, 413 aa, Homo sapiens [sequence omitted]